European Patent Application EP 4 375 375 A1, published May 29, 2024. Title: がん患者の予後を予測するためのバイオマーカー、がん患者の予後を予測するための方法、がん患者における、がん治療薬の効果を予測するための方法、及び、がん患者の予後を予測するためのキット. Applicant: 国立大学法人東北大学. The sequence listing filed with the application follows.

SEQUENCE LISTING (10 sequences)

SEQ ID NO: 1 - protein, 258 aa, Homo sapiens
MIPTFTALLCLGLSLGPRTHMQAGPLPKPTLWAEPGSVISWGNSVTIWCQGTLEAREYRLDKEESPAPWDRQNPLEPKNKARFSIPSMTEDYAGRYRCYYRSPVGWSQPSDPLELVMTGAYSKPTLSALPSPLVTSGKSVTLLCQSRSPMDTFLLIKERAAHPLLHLRSEHGAQQHQAEFPMSPVTSVHGGTYRCFSSHGFSHYLLSHPSDPLELIVSGSLEDPRPSPTRSVSTAAGPEDQPLMPTGSVPHSGLRRHW

SEQ ID NO: 2 - protein, 20 aa, Homo sapiens
CTCIGAGRGRISCTIANRCH

SEQ ID NO: 3 - protein, 10 aa, Mus musculus
GFTFSSFGMH

SEQ ID NO: 4 - protein, 17 aa, Mus musculus
YISSGSSTIYYVDTVKG

SEQ ID NO: 5 - protein, 9 aa, Mus musculus
STGTGAMDY

SEQ ID NO: 6 - protein, 11 aa, Mus musculus
RASQDISNYLN

SEQ ID NO: 7 - protein, 7 aa, Mus musculus
YTLRLYS

SEQ ID NO: 8 - protein, 9 aa, Mus musculus
QQGNTLPWT

SEQ ID NO: 9 - protein, 118 aa, Mus musculus
EVMLVESGGGLVQPGGSRKLSCAASGFTFSSFGMHWVRQAPEKGLEWVAYISSGSSTIYYVDTVKGRFTISRDNPKNTLFLQMTSLRSEDTAMYYCARSTGTGAMDYWGQGTSVTVSS

SEQ ID NO: 10 - protein, 107 aa, Mus musculus
DIQMTQTTSSLSASLGDRVTISCRASQDISNYLNWYQQKPDGTVKLLIYYTLRLYSGVPSRFSGSGSGTDYSLTISNLEQEDIATYFCQQGNTLPWTFGGGTKLEIK